European Patent Specification EP 3 797 776 B1, published July 23, 2025. Title: Agent for the treatment of psoriasis. Applicant: Eberhard-Karls-Universität Medizinische Fakultät. The sequence listing filed with the application follows.

SEQUENCE LISTING (8 sequences)

SEQ ID NO: 1 - DNA, 25 bp, Artificial Sequence
  Guide RNA
caccgactgctggtcaatctctccc

SEQ ID NO: 2 - DNA, 25 bp, Artificial Sequence
  Guide RNA
aaacgggagagattgaccagcagtc

SEQ ID NO: 3 - protein, 16 aa, Artificial Sequence
  Epitope
CSAPGSPGSDSSDFSS

SEQ ID NO: 4 - protein, 14 aa, Artificial Sequence
  Epitope
CLHIRSHKQKASGQ

SEQ ID NO: 5 - DNA, 20 bp, Artificial Sequence
  Promoter
ctctgctcctttgccacaac

SEQ ID NO: 6 - DNA, 20 bp, Artificial Sequence
  Promoter
gagtgctcttcgggtttcag

SEQ ID NO: 7 - DNA, 20 bp, Artificial Sequence
  Promoter
gccttaactgggctaacagc

SEQ ID NO: 8 - DNA, 20 bp, Artificial Sequence
  Promoter
ctggcaagtcctggaaggag